European Patent Specification EP 3 597 741 B1, published June 3, 2026. Title: GENETIC CORRECTION OF MUTATED GENES. Applicant: DUKE UNIVERSITY. Application not yet assigned. The sequence listing filed with the application follows.

SEQUENCE LISTING (93 sequences)

SEQ ID NO: 1 - protein, 976 aa, Artificial Sequence
  Synthetic
MDYKDHDGDYKDHDIDYKDDDDKMAPKKKRKVGRGSVRSTVAQHHEALVGHGFTHAHIVALSQHPAALGTVAVTYQHIITALPEATHEDIVGVGKQWSGARALEALLTDAGELRGPPLQLDTGQLVKIAKRGGVTAMEAVHASRNALTGAPLNLTPDQVVAIASNGGGKQALETVQRLLPVLCQDHGLTPDQVVAIASNGGGKQALETVQRLLPVLCQDHGLTPDQVVAIASNGGGKQALETVQRLLPVLCQDHGLTPDQVVAIASNIGGKQALETVQRLLPVLCQDHGLTPDQVVAIASNNGGKQALETVQRLLPVLCQDHGLTPDQVVAIASHDGGKQALETVQRLLPVLCQDHGLTPDQVVAIASNGGGKQALETVQRLLPVLCQDHGLTPDQVVAIASHDGGKQALETVQRLLPVLCQDHGLTPDQVVAIASHDGGKQALETVQRLLPVLCQDHGLTPDQVVAIASNGGGKQALETVQRLLPVLCQDHGLTPDQVVAIASNIGGKQALETVQRLLPVLCQDHGLTPDQVVAIASHDGGKQALETVQRLLPVLCQDHGLTPDQVVAIASNGGGKQALETVQRLLPVLCQDHGLTPDQVVAIASHDGGKQALETVQRLLPVLCQDHGLTPDQVVAIASNIGGKQALETVQRLLPVLCQDHGLTPDQVVAIASNNGGKQALETVQRLLPVLCQDHGLTPDQVVAIASNIGGKQALESIVAQLSRPDPALAALTNDHLVALACLGGRPAMDAVKKGLPHAPELIRRVNRRIGERTSHRVAQLVKSELEEKKSELRHKLKYVPHEYIELIEIARNPTQDRILEMKVMEFFMKVYGYRGEHLGGSRKPDGAIYTVGSPIDYGVIVDTKAYSGGYNLPIGQADEMERYVEENQTRDKHLNPNEWWKVYPSSVTEFKFLFVSGHFKGNYKAQLTRLNHITNCNGAVLSVEELLIGGEMIKAGTLTLEEVRRKFNNGEINF

SEQ ID NO: 2 - protein, 942 aa, Artificial Sequence
  Synthetic
MDYKDHDGDYKDHDIDYKDDDDKMAPKKKRKVGRGSVRSTVAQHHEALVGHGFTHAHIVALSQHPAALGTVAVTYQHIITALPEATHEDIVGVGKQWSGARALEALLTDAGELRGPPLQLDTGQLVKIAKRGGVTAMEAVHASRNALTGAPLNLTPDQVVAIASNIGGKQALETVQRLLPVLCQDHGLTPDQVVAIASNNGGKQALETVQRLLPVLCQDHGLTPDQVVAIASHDGGKQALETVQRLLPVLCQDHGLTPDQVVAIASNGGGKQALETVQRLLPVLCQDHGLTPDQVVAIASHDGGKQALETVQRLLPVLCQDHGLTPDQVVAIASHDGGKQALETVQRLLPVLCQDHGLTPDQVVAIASNGGGKQALETVQRLLPVLCQDHGLTPDQVVAIASNIGGKQALETVQRLLPVLCQDHGLTPDQVVAIASHDGGKQALETVQRLLPVLCQDHGLTPDQVVAIASNGGGKQALETVQRLLPVLCQDHGLTPDQVVAIASHDGGKQALETVQRLLPVLCQDHGLTPDQVVAIASNIGGKQALETVQRLLPVLCQDHGLTPDQVVAIASNNGGKQALETVQRLLPVLCQDHGLTPDQVVAIASNIGGKQALETVQRLLPVLCQDHGLTPDQVVAIASHDGGKQALETVQRLLPVLCQDHGLTPDQVVAIASNGGGKQALESIVAQLSRPDPALAALTNDHLVALACLGGRPAMDAVKKGLPHAPELIRRVNRRIGERTSHRVAQLVKSELEEKKSELRHKLKYVPHEYIELIEIARNPTQDRILEMKVMEFFMKVYGYRGEHLGGSRKPDGAIYTVGSPIDYGVIVDTKAYSGGYNLPIGQADEMERYVEENQTRDKHLNPNEWWKVYPSSVTEFKFLFVSGHFKGNYKAQLTRLNHITNCNGAVLSVEELLIGGEMIKAGTLTLEEVRRKFNNGEINF

SEQ ID NO: 3 - protein, 942 aa, Artificial Sequence
  Synthetic
MDYKDHDGDYKDHDIDYKDDDDKMAPKKKRKVGRGSVRSTVAQHHEALVGHGFTHAHIVALSQHPAALGTVAVTYQHIITALPEATHEDIVGVGKQWSGARALEALLTDAGELRGPPLQLDTGQLVKIAKRGGVTAMEAVHASRNALTGAPLNLTPDQVVAIASNIGGKQALETVQRLLPVLCQDHGLTPDQVVAIASNNGGKQALETVQRLLPVLCQDHGLTPDQVVAIASNGGGKQALETVQRLLPVLCQDHGLTPDQVVAIASNIGGKQALETVQRLLPVLCQDHGLTPDQVVAIASNIGGKQALETVQRLLPVLCQDHGLTPDQVVAIASHDGGKQALETVQRLLPVLCQDHGLTPDQVVAIASHDGGKQALETVQRLLPVLCQDHGLTPDQVVAIASNIGGKQALETVQRLLPVLCQDHGLTPDQVVAIASHDGGKQALETVQRLLPVLCQDHGLTPDQVVAIASNIGGKQALETVQRLLPVLCQDHGLTPDQVVAIASNNGGKQALETVQRLLPVLCQDHGLTPDQVVAIASNNGGKQALETVQRLLPVLCQDHGLTPDQVVAIASNGGGKQALETVQRLLPVLCQDHGLTPDQVVAIASNGGGKQALETVQRLLPVLCQDHGLTPDQVVAIASNNGGKQALETVQRLLPVLCQDHGLTPDQVVAIASNGGGKQALESIVAQLSRPDPALAALTNDHLVALACLGGRPAMDAVKKGLPHAPELIRRVNRRIGERTSHRVAQLVKSELEEKKSELRHKLKYVPHEYIELIEIARNPTQDRILEMKVMEFFMKVYGYRGEHLGGSRKPDGAIYTVGSPIDYGVIVDTKAYSGGYNLPIGQADEMQRYVKENQTRNKHINPNEWWKVYPSSVTEFKFLFVSGHFKGNYKAQLTRLNRKTNCNGAVLSVEELLIGGEMIKAGTLTLEEVRRKFNNGEINF

SEQ ID NO: 4 - protein, 976 aa, Artificial Sequence
  Synthetic
MDYKDHDGDYKDHDIDYKDDDDKMAPKKKRKVGRGSVRSTVAQHHEALVGHGFTHAHIVALSQHPAALGTVAVTYQHIITALPEATHEDIVGVGKQWSGARALEALLTDAGELRGPPLQLDTGQLVKIAKRGGVTAMEAVHASRNALTGAPLNLTPDQVVAIASHDGGKQALETVQRLLPVLCQDHGLTPDQVVAIASHDGGKQALETVQRLLPVLCQDHGLTPDQVVAIASNGGGKQALETVQRLLPVLCQDHGLTPDQVVAIASNGGGKQALETVQRLLPVLCQDHGLTPDQVVAIASNIGGKQALETVQRLLPVLCQDHGLTPDQVVAIASNNGGKQALETVQRLLPVLCQDHGLTPDQVVAIASNGGGKQALETVQRLLPVLCQDHGLTPDQVVAIASNIGGKQALETVQRLLPVLCQDHGLTPDQVVAIASNIGGKQALETVQRLLPVLCQDHGLTPDQVVAIASHDGGKQALETVQRLLPVLCQDHGLTPDQVVAIASHDGGKQALETVQRLLPVLCQDHGLTPDQVVAIASNIGGKQALETVQRLLPVLCQDHGLTPDQVVAIASHDGGKQALETVQRLLPVLCQDHGLTPDQVVAIASNIGGKQALETVQRLLPVLCQDHGLTPDQVVAIASNNGGKQALETVQRLLPVLCQDHGLTPDQVVAIASNNGGKQALETVQRLLPVLCQDHGLTPDQVVAIASNGGGKQALESIVAQLSRPDPALAALTNDHLVALACLGGRPAMDAVKKGLPHAPELIRRVNRRIGERTSHRVAQLVKSELEEKKSELRHKLKYVPHEYIELIEIARNPTQDRILEMKVMEFFMKVYGYRGEHLGGSRKPDGAIYTVGSPIDYGVIVDTKAYSGGYNLPIGQADEMQRYVKENQTRNKHINPNEWWKVYPSSVTEFKFLFVSGHFKGNYKAQLTRLNRKTNCNGAVLSVEELLIGGEMIKAGTLTLEEVRRKFNNGEINF

SEQ ID NO: 5 - protein, 976 aa, Artificial Sequence
  Synthetic
MDYKDHDGDYKDHDIDYKDDDDKMAPKKKRKVGRGSVRSTVAQHHEALVGHGFTHAHIVALSQHPAALGTVAVTYQHIITALPEATHEDIVGVGKQWSGARALEALLTDAGELRGPPLQLDTGQLVKIAKRGGVTAMEAVHASRNALTGAPLNLTPDQVVAIASNNGGKQALETVQRLLPVLCQDHGLTPDQVVAIASHDGGKQALETVQRLLPVLCQDHGLTPDQVVAIASNIGGKQALETVQRLLPVLCQDHGLTPDQVVAIASNIGGKQALETVQRLLPVLCQDHGLTPDQVVAIASNIGGKQALETVQRLLPVLCQDHGLTPDQVVAIASNIGGKQALETVQRLLPVLCQDHGLTPDQVVAIASNIGGKQALETVQRLLPVLCQDHGLTPDQVVAIASHDGGKQALETVQRLLPVLCQDHGLTPDQVVAIASHDGGKQALETVQRLLPVLCQDHGLTPDQVVAIASHDGGKQALETVQRLLPVLCQDHGLTPDQVVAIASNIGGKQALETVQRLLPVLCQDHGLTPDQVVAIASNIGGKQALETVQRLLPVLCQDHGLTPDQVVAIASNIGGKQALETVQRLLPVLCQDHGLTPDQVVAIASNIGGKQALETVQRLLPVLCQDHGLTPDQVVAIASNGGGKQALETVQRLLPVLCQDHGLTPDQVVAIASNIGGKQALETVQRLLPVLCQDHGLTPDQVVAIASNGGGKQALESIVAQLSRPDPALAALTNDHLVALACLGGRPAMDAVKKGLPHAPELIRRVNRRIGERTSHRVAQLVKSELEEKKSELRHKLKYVPHEYIELIEIARNPTQDRILEMKVMEFFMKVYGYRGEHLGGSRKPDGAIYTVGSPIDYGVIVDTKAYSGGYNLPIGQADEMERYVEENQTRDKHLNPNEWWKVYPSSVTEFKFLFVSGHFKGNYKAQLTRLNHITNCNGAVLSVEELLIGGEMIKAGTLTLEEVRRKFNNGEINF

SEQ ID NO: 6 - protein, 976 aa, Artificial Sequence
  Synthetic
MDYKDHDGDYKDHDIDYKDDDDKMAPKKKRKVGRGSVRSTVAQHHEALVGHGFTHAHIVALSQHPAALGTVAVTYQHIITALPEATHEDIVGVGKQWSGARALEALLTDAGELRGPPLQLDTGQLVKIAKRGGVTAMEAVHASRNALTGAPLNLTPDQVVAIASNGGGKQALETVQRLLPVLCQDHGLTPDQVVAIASNGGGKQALETVQRLLPVLCQDHGLTPDQVVAIASNNGGKQALETVQRLLPVLCQDHGLTPDQVVAIASHDGGKQALETVQRLLPVLCQDHGLTPDQVVAIASNIGGKQALETVQRLLPVLCQDHGLTPDQVVAIASNIGGKQALETVQRLLPVLCQDHGLTPDQVVAIASNIGGKQALETVQRLLPVLCQDHGLTPDQVVAIASNIGGKQALETVQRLLPVLCQDHGLTPDQVVAIASNIGGKQALETVQRLLPVLCQDHGLTPDQVVAIASHDGGKQALETVQRLLPVLCQDHGLTPDQVVAIASHDGGKQALETVQRLLPVLCQDHGLTPDQVVAIASHDGGKQALETVQRLLPVLCQDHGLTPDQVVAIASNIGGKQALETVQRLLPVLCQDHGLTPDQVVAIASNIGGKQALETVQRLLPVLCQDHGLTPDQVVAIASNIGGKQALETVQRLLPVLCQDHGLTPDQVVAIASNIGGKQALETVQRLLPVLCQDHGLTPDQVVAIASNGGGKQALESIVAQLSRPDPALAALTNDHLVALACLGGRPAMDAVKKGLPHAPELIRRVNRRIGERTSHRVAQLVKSELEEKKSELRHKLKYVPHEYIELIEIARNPTQDRILEMKVMEFFMKVYGYRGEHLGGSRKPDGAIYTVGSPIDYGVIVDTKAYSGGYNLPIGQADEMERYVEENQTRDKHLNPNEWWKVYPSSVTEFKFLFVSGHFKGNYKAQLTRLNHITNCNGAVLSVEELLIGGEMIKAGTLTLEEVRRKFNNGEINF

SEQ ID NO: 7 - protein, 976 aa, Artificial Sequence
  Synthetic
MDYKDHDGDYKDHDIDYKDDDDKMAPKKKRKVGRGSVRSTVAQHHEALVGHGFTHAHIVALSQHPAALGTVAVTYQHIITALPEATHEDIVGVGKQWSGARALEALLTDAGELRGPPLQLDTGQLVKIAKRGGVTAMEAVHASRNALTGAPLNLTPDQVVAIASHDGGKQALETVQRLLPVLCQDHGLTPDQVVAIASHDGGKQALETVQRLLPVLCQDHGLTPDQVVAIASNGGGKQALETVQRLLPVLCQDHGLTPDQVVAIASNGGGKQALETVQRLLPVLCQDHGLTPDQVVAIASNGGGKQALETVQRLLPVLCQDHGLTPDQVVAIASNGGGKQALETVQRLLPVLCQDHGLTPDQVVAIASNGGGKQALETVQRLLPVLCQDHGLTPDQVVAIASNNGGKQALETVQRLLPVLCQDHGLTPDQVVAIASHDGGKQALETVQRLLPVLCQDHGLTPDQVVAIASNIGGKQALETVQRLLPVLCQDHGLTPDQVVAIASNIGGKQALETVQRLLPVLCQDHGLTPDQVVAIASNIGGKQALETVQRLLPVLCQDHGLTPDQVVAIASNIGGKQALETVQRLLPVLCQDHGLTPDQVVAIASNIGGKQALETVQRLLPVLCQDHGLTPDQVVAIASHDGGKQALETVQRLLPVLCQDHGLTPDQVVAIASHDGGKQALETVQRLLPVLCQDHGLTPDQVVAIASHDGGKQALESIVAQLSRPDPALAALTNDHLVALACLGGRPAMDAVKKGLPHAPELIRRVNRRIGERTSHRVAQLVKSELEEKKSELRHKLKYVPHEYIELIEIARNPTQDRILEMKVMEFFMKVYGYRGEHLGGSRKPDGAIYTVGSPIDYGVIVDTKAYSGGYNLPIGQADEMERYVEENQTRDKHLNPNEWWKVYPSSVTEFKFLFVSGHFKGNYKAQLTRLNHITNCNGAVLSVEELLIGGEMIKAGTLTLEEVRRKFNNGEINF

SEQ ID NO: 8 - protein, 976 aa, Artificial Sequence
  Synthetic
MDYKDHDGDYKDHDIDYKDDDDKMAPKKKRKVGRGSVRSTVAQHHEALVGHGFTHAHIVALSQHPAALGTVAVTYQHIITALPEATHEDIVGVGKQWSGARALEALLTDAGELRGPPLQLDTGQLVKIAKRGGVTAMEAVHASRNALTGAPLNLTPDQVVAIASHDGGKQALETVQRLLPVLCQDHGLTPDQVVAIASNIGGKQALETVQRLLPVLCQDHGLTPDQVVAIASHDGGKQALETVQRLLPVLCQDHGLTPDQVVAIASHDGGKQALETVQRLLPVLCQDHGLTPDQVVAIASNIGGKQALETVQRLLPVLCQDHGLTPDQVVAIASNNGGKQALETVQRLLPVLCQDHGLTPDQVVAIASNIGGKQALETVQRLLPVLCQDHGLTPDQVVAIASNNGGKQALETVQRLLPVLCQDHGLTPDQVVAIASNGGGKQALETVQRLLPVLCQDHGLTPDQVVAIASNIGGKQALETVQRLLPVLCQDHGLTPDQVVAIASNIGGKQALETVQRLLPVLCQDHGLTPDQVVAIASHDGGKQALETVQRLLPVLCQDHGLTPDQVVAIASNIGGKQALETVQRLLPVLCQDHGLTPDQVVAIASNNGGKQALETVQRLLPVLCQDHGLTPDQVVAIASNGGGKQALETVQRLLPVLCQDHGLTPDQVVAIASHDGGKQALETVQRLLPVLCQDHGLTPDQVVAIASNGGGKQALESIVAQLSRPDPALAALTNDHLVALACLGGRPAMDAVKKGLPHAPELIRRVNRRIGERTSHRVAQLVKSELEEKKSELRHKLKYVPHEYIELIEIARNPTQDRILEMKVMEFFMKVYGYRGEHLGGSRKPDGAIYTVGSPIDYGVIVDTKAYSGGYNLPIGQADEMQRYVKENQTRNKHINPNEWWKVYPSSVTEFKFLFVSGHFKGNYKAQLTRLNRKTNCNGAVLSVEELLIGGEMIKAGTLTLEEVRRKFNNGEINF

SEQ ID NO: 9 - protein, 1044 aa, Artificial Sequence
  Synthetic
MDYKDHDGDYKDHDIDYKDDDDKMAPKKKRKVGRGSVRSTVAQHHEALVGHGFTHAHIVALSQHPAALGTVAVTYQHIITALPEATHEDIVGVGKQWSGARALEALLTDAGELRGPPLQLDTGQLVKIAKRGGVTAMEAVHASRNALTGAPLNLTPDQVVAIASNNGGKQALETVQRLLPVLCQDHGLTPDQVVAIASNGGGKQALETVQRLLPVLCQDHGLTPDQVVAIASHDGGKQALETVQRLLPVLCQDHGLTPDQVVAIASNIGGKQALETVQRLLPVLCQDHGLTPDQVVAIASHDGGKQALETVQRLLPVLCQDHGLTPDQVVAIASHDGGKQALETVQRLLPVLCQDHGLTPDQVVAIASNIGGKQALETVQRLLPVLCQDHGLTPDQVVAIASNNGGKQALETVQRLLPVLCQDHGLTPDQVVAIASNIGGKQALETVQRLLPVLCQDHGLTPDQVVAIASNNGGKQALETVQRLLPVLCQDHGLTPDQVVAIASNGGGKQALETVQRLLPVLCQDHGLTPDQVVAIASNIGGKQALETVQRLLPVLCQDHGLTPDQVVAIASNIGGKQALETVQRLLPVLCQDHGLTPDQVVAIASHDGGKQALETVQRLLPVLCQDHGLTPDQVVAIASNIGGKQALETVQRLLPVLCQDHGLTPDQVVAIASNNGGKQALETVQRLLPVLCQDHGLTPDQVVAIASNGGGKQALETVQRLLPVLCQDHGLTPDQVVAIASHDGGKQALETVQRLLPVLCQDHGLTPDQVVAIASNGGGKQALESIVAQLSRPDPALAALTNDHLVALACLGGRPAMDAVKKGLPHAPELIRRVNRRIGERTSHRVAQLVKSELEEKKSELRHKLKYVPHEYIELIEIARNPTQDRILEMKVMEFFMKVYGYRGEHLGGSRKPDGAIYTVGSPIDYGVIVDTKAYSGGYNLPIGQADEMQRYVKENQTRNKHINPNEWWKVYPSSVTEFKFLFVSGHFKGNYKAQLTRLNRKTNCNGAVLSVEELLIGGEMIKAGTLTLEEVRRKFNNGEINF

SEQ ID NO: 10 - protein, 1044 aa, Artificial Sequence
  Synthetic
MDYKDHDGDYKDHDIDYKDDDDKMAPKKKRKVGRGSVRSTVAQHHEALVGHGFTHAHIVALSQHPAALGTVAVTYQHIITALPEATHEDIVGVGKQWSGARALEALLTDAGELRGPPLQLDTGQLVKIAKRGGVTAMEAVHASRNALTGAPLNLTPDQVVAIASHDGGKQALETVQRLLPVLCQDHGLTPDQVVAIASNGGGKQALETVQRLLPVLCQDHGLTPDQVVAIASNGGGKQALETVQRLLPVLCQDHGLTPDQVVAIASHDGGKQALETVQRLLPVLCQDHGLTPDQVVAIASHDGGKQALETVQRLLPVLCQDHGLTPDQVVAIASNGGGKQALETVQRLLPVLCQDHGLTPDQVVAIASNGGGKQALETVQRLLPVLCQDHGLTPDQVVAIASNNGGKQALETVQRLLPVLCQDHGLTPDQVVAIASNIGGKQALETVQRLLPVLCQDHGLTPDQVVAIASNGGGKQALETVQRLLPVLCQDHGLTPDQVVAIASNNGGKQALETVQRLLPVLCQDHGLTPDQVVAIASNGGGKQALETVQRLLPVLCQDHGLTPDQVVAIASNGGGKQALETVQRLLPVLCQDHGLTPDQVVAIASNNGGKQALETVQRLLPVLCQDHGLTPDQVVAIASNNGGKQALETVQRLLPVLCQDHGLTPDQVVAIASNIGGKQALETVQRLLPVLCQDHGLTPDQVVAIASNNGGKQALETVQRLLPVLCQDHGLTPDQVVAIASNNGGKQALETVQRLLPVLCQDHGLTPDQVVAIASNGGGKQALESIVAQLSRPDPALAALTNDHLVALACLGGRPAMDAVKKGLPHAPELIRRVNRRIGERTSHRVAQLVKSELEEKKSELRHKLKYVPHEYIELIEIARNPTQDRILEMKVMEFFMKVYGYRGEHLGGSRKPDGAIYTVGSPIDYGVIVDTKAYSGGYNLPIGQADEMERYVEENQTRDKHLNPNEWWKVYPSSVTEFKFLFVSGHFKGNYKAQLTRLNHITNCNGAVLSVEELLIGGEMIKAGTLTLEEVRRKFNNGEINF

SEQ ID NO: 11 - protein, 1044 aa, Artificial Sequence
  Synthetic
MDYKDHDGDYKDHDIDYKDDDDKMAPKKKRKVGRGSVRSTVAQHHEALVGHGFTHAHIVALSQHPAALGTVAVTYQHIITALPEATHEDIVGVGKQWSGARALEALLTDAGELRGPPLQLDTGQLVKIAKRGGVTAMEAVHASRNALTGAPLNLTPDQVVAIASNIGGKQALETVQRLLPVLCQDHGLTPDQVVAIASHDGGKQALETVQRLLPVLCQDHGLTPDQVVAIASHDGGKQALETVQRLLPVLCQDHGLTPDQVVAIASNGGGKQALETVQRLLPVLCQDHGLTPDQVVAIASNNGGKQALETVQRLLPVLCQDHGLTPDQVVAIASHDGGKQALETVQRLLPVLCQDHGLTPDQVVAIASNGGGKQALETVQRLLPVLCQDHGLTPDQVVAIASHDGGKQALETVQRLLPVLCQDHGLTPDQVVAIASNGGGKQALETVQRLLPVLCQDHGLTPDQVVAIASNNGGKQALETVQRLLPVLCQDHGLTPDQVVAIASNNGGKQALETVQRLLPVLCQDHGLTPDQVVAIASHDGGKQALETVQRLLPVLCQDHGLTPDQVVAIASNIGGKQALETVQRLLPVLCQDHGLTPDQVVAIASNNGGKQALETVQRLLPVLCQDHGLTPDQVVAIASNIGGKQALETVQRLLPVLCQDHGLTPDQVVAIASNGGGKQALETVQRLLPVLCQDHGLTPDQVVAIASNGGGKQALETVQRLLPVLCQDHGLTPDQVVAIASNGGGKQALETVQRLLPVLCQDHGLTPDQVVAIASHDGGKQALESIVAQLSRPDPALAALTNDHLVALACLGGRPAMDAVKKGLPHAPELIRRVNRRIGERTSHRVAQLVKSELEEKKSELRHKLKYVPHEYIELIEIARNPTQDRILEMKVMEFFMKVYGYRGEHLGGSRKPDGAIYTVGSPIDYGVIVDTKAYSGGYNLPIGQADEMQRYVKENQTRNKHINPNEWWKVYPSSVTEFKFLFVSGHFKGNYKAQLTRLNRKTNCNGAVLSVEELLIGGEMIKAGTLTLEEVRRKFNNGEINF

SEQ ID NO: 12 - protein, 1010 aa, Artificial Sequence
  Synthetic
MDYKDHDGDYKDHDIDYKDDDDKMAPKKKRKVGRGSVRSTVAQHHEALVGHGFTHAHIVALSQHPAALGTVAVTYQHIITALPEATHEDIVGVGKQWSGARALEALLTDAGELRGPPLQLDTGQLVKIAKRGGVTAMEAVHASRNALTGAPLNLTPDQVVAIASHDGGKQALETVQRLLPVLCQDHGLTPDQVVAIASNGGGKQALETVQRLLPVLCQDHGLTPDQVVAIASNIGGKQALETVQRLLPVLCQDHGLTPDQVVAIASNGGGKQALETVQRLLPVLCQDHGLTPDQVVAIASNIGGKQALETVQRLLPVLCQDHGLTPDQVVAIASNNGGKQALETVQRLLPVLCQDHGLTPDQVVAIASNIGGKQALETVQRLLPVLCQDHGLTPDQVVAIASNGGGKQALETVQRLLPVLCQDHGLTPDQVVAIASNNGGKQALETVQRLLPVLCQDHGLTPDQVVAIASNIGGKQALETVQRLLPVLCQDHGLTPDQVVAIASNNGGKQALETVQRLLPVLCQDHGLTPDQVVAIASNIGGKQALETVQRLLPVLCQDHGLTPDQVVAIASNGGGKQALETVQRLLPVLCQDHGLTPDQVVAIASNGGGKQALETVQRLLPVLCQDHGLTPDQVVAIASNIGGKQALETVQRLLPVLCQDHGLTPDQVVAIASNGGGKQALETVQRLLPVLCQDHGLTPDQVVAIASHDGGKQALETVQRLLPVLCQDHGLTPDQVVAIASNGGGKQALESIVAQLSRPDPALAALTNDHLVALACLGGRPAMDAVKKGLPHAPELIRRVNRRIGERTSHRVAQLVKSELEEKKSELRHKLKYVPHEYIELIEIARNPTQDRILEMKVMEFFMKVYGYRGEHLGGSRKPDGAIYTVGSPIDYGVIVDTKAYSGGYNLPIGQADEMERYVEENQTRDKHLNPNEWWKVYPSSVTEFKFLFVSGHFKGNYKAQLTRLNHITNCNGAVLSVEELLIGGEMIKAGTLTLEEVRRKFNNGEINF

SEQ ID NO: 13 - protein, 1010 aa, Artificial Sequence
  Synthetic
MDYKDHDGDYKDHDIDYKDDDDKMAPKKKRKVGRGSVRSTVAQHHEALVGHGFTHAHIVALSQHPAALGTVAVTYQHIITALPEATHEDIVGVGKQWSGARALEALLTDAGELRGPPLQLDTGQLVKIAKRGGVTAMEAVHASRNALTGAPLNLTPDQVVAIASNIGGKQALETVQRLLPVLCQDHGLTPDQVVAIASNNGGKQALETVQRLLPVLCQDHGLTPDQVVAIASHDGGKQALETVQRLLPVLCQDHGLTPDQVVAIASNIGGKQALETVQRLLPVLCQDHGLTPDQVVAIASNIGGKQALETVQRLLPVLCQDHGLTPDQVVAIASNGGGKQALETVQRLLPVLCQDHGLTPDQVVAIASNNGGKQALETVQRLLPVLCQDHGLTPDQVVAIASHDGGKQALETVQRLLPVLCQDHGLTPDQVVAIASNNGGKQALETVQRLLPVLCQDHGLTPDQVVAIASNNGGKQALETVQRLLPVLCQDHGLTPDQVVAIASHDGGKQALETVQRLLPVLCQDHGLTPDQVVAIASHDGGKQALETVQRLLPVLCQDHGLTPDQVVAIASNIGGKQALETVQRLLPVLCQDHGLTPDQVVAIASNGGGKQALETVQRLLPVLCQDHGLTPDQVVAIASHDGGKQALETVQRLLPVLCQDHGLTPDQVVAIASHDGGKQALETVQRLLPVLCQDHGLTPDQVVAIASHDGGKQALETVQRLLPVLCQDHGLTPDQVVAIASNGGGKQALESIVAQLSRPDPALAALTNDHLVALACLGGRPAMDAVKKGLPHAPELIRRVNRRIGERTSHRVAQLVKSELEEKKSELRHKLKYVPHEYIELIEIARNPTQDRILEMKVMEFFMKVYGYRGEHLGGSRKPDGAIYTVGSPIDYGVIVDTKAYSGGYNLPIGQADEMQRYVKENQTRNKHINPNEWWKVYPSSVTEFKFLFVSGHFKGNYKAQLTRLNRKTNCNGAVLSVEELLIGGEMIKAGTLTLEEVRRKFNNGEINF

SEQ ID NO: 14 - protein, 942 aa, Artificial Sequence
  Synthetic
MDYKDHDGDYKDHDIDYKDDDDKMAPKKKRKVGRGSVRSTVAQHHEALVGHGFTHAHIVALSQHPAALGTVAVTYQHIITALPEATHEDIVGVGKQWSGARALEALLTDAGELRGPPLQLDTGQLVKIAKRGGVTAMEAVHASRNALTGAPLNLTPDQVVAIASNIGGKQALETVQRLLPVLCQDHGLTPDQVVAIASNIGGKQALETVQRLLPVLCQDHGLTPDQVVAIASHDGGKQALETVQRLLPVLCQDHGLTPDQVVAIASNGGGKQALETVQRLLPVLCQDHGLTPDQVVAIASNNGGKQALETVQRLLPVLCQDHGLTPDQVVAIASNIGGKQALETVQRLLPVLCQDHGLTPDQVVAIASNGGGKQALETVQRLLPVLCQDHGLTPDQVVAIASNNGGKQALETVQRLLPVLCQDHGLTPDQVVAIASHDGGKQALETVQRLLPVLCQDHGLTPDQVVAIASHDGGKQALETVQRLLPVLCQDHGLTPDQVVAIASNIGGKQALETVQRLLPVLCQDHGLTPDQVVAIASNNGGKQALETVQRLLPVLCQDHGLTPDQVVAIASNNGGKQALETVQRLLPVLCQDHGLTPDQVVAIASNIGGKQALETVQRLLPVLCQDHGLTPDQVVAIASNGGGKQALETVQRLLPVLCQDHGLTPDQVVAIASNGGGKQALESIVAQLSRPDPALAALTNDHLVALACLGGRPAMDAVKKGLPHAPELIRRVNRRIGERTSHRVAQLVKSELEEKKSELRHKLKYVPHEYIELIEIARNPTQDRILEMKVMEFFMKVYGYRGEHLGGSRKPDGAIYTVGSPIDYGVIVDTKAYSGGYNLPIGQADEMQRYVKENQTRNKHINPNEWWKVYPSSVTEFKFLFVSGHFKGNYKAQLTRLNRKTNCNGAVLSVEELLIGGEMIKAGTLTLEEVRRKFNNGEINF

SEQ ID NO: 15 - protein, 942 aa, Artificial Sequence
  Synthetic
MDYKDHDGDYKDHDIDYKDDDDKMAPKKKRKVGRGSVRSTVAQHHEALVGHGFTHAHIVALSQHPAALGTVAVTYQHIITALPEATHEDIVGVGKQWSGARALEALLTDAGELRGPPLQLDTGQLVKIAKRGGVTAMEAVHASRNALTGAPLNLTPDQVVAIASNNGGKQALETVQRLLPVLCQDHGLTPDQVVAIASNNGGKQALETVQRLLPVLCQDHGLTPDQVVAIASNIGGKQALETVQRLLPVLCQDHGLTPDQVVAIASNIGGKQALETVQRLLPVLCQDHGLTPDQVVAIASNGGGKQALETVQRLLPVLCQDHGLTPDQVVAIASNGGGKQALETVQRLLPVLCQDHGLTPDQVVAIASNGGGKQALETVQRLLPVLCQDHGLTPDQVVAIASNNGGKQALETVQRLLPVLCQDHGLTPDQVVAIASNIGGKQALETVQRLLPVLCQDHGLTPDQVVAIASNIGGKQALETVQRLLPVLCQDHGLTPDQVVAIASNIGGKQALETVQRLLPVLCQDHGLTPDQVVAIASNGGGKQALETVQRLLPVLCQDHGLTPDQVVAIASNIGGKQALETVQRLLPVLCQDHGLTPDQVVAIASNGGGKQALETVQRLLPVLCQDHGLTPDQVVAIASHDGGKQALETVQRLLPVLCQDHGLTPDQVVAIASHDGGKQALESIVAQLSRPDPALAALTNDHLVALACLGGRPAMDAVKKGLPHAPELIRRVNRRIGERTSHRVAQLVKSELEEKKSELRHKLKYVPHEYIELIEIARNPTQDRILEMKVMEFFMKVYGYRGEHLGGSRKPDGAIYTVGSPIDYGVIVDTKAYSGGYNLPIGQADEMERYVEENQTRDKHLNPNEWWKVYPSSVTEFKFLFVSGHFKGNYKAQLTRLNHITNCNGAVLSVEELLIGGEMIKAGTLTLEEVRRKFNNGEINF

SEQ ID NO: 16 - DNA, 49 bp, Homo sapiens
tttagctcctactcagactgttactctggtgacacaacctgtggttact

SEQ ID NO: 17 - DNA, 53 bp, Homo sapiens
tttagctcctactcagactgttactctggtgacacaacctgtggttactaagg

SEQ ID NO: 18 - DNA, 46 bp, Homo sapiens
agctcctactcagactgttactctggtgacacaacctgtggttact

SEQ ID NO: 19 - DNA, 50 bp, Homo sapiens
agctcctactcagactgttactctggtgacacaacctgtggttactaagg

SEQ ID NO: 20 - DNA, 50 bp, Homo sapiens
gcaaaaacccaaaatattttagctcctactcagactgttactctggtgac

SEQ ID NO: 21 - DNA, 52 bp, Homo sapiens
ttgcaaaaacccaaaatattttagctcctactcagactgttactctggtgac

SEQ ID NO: 22 - DNA, 55 bp, Homo sapiens
cctttttgcaaaaacccaaaatattttagctcctactcagactgttactctggtg

SEQ ID NO: 23 - DNA, 56 bp, Homo sapiens
ccaaactagaaatgccatcttccttgatgttggaggtacctgctctggcagatttc

SEQ ID NO: 24 - DNA, 51 bp, Homo sapiens
ctatagatgagattatctgcccatgactggcgcagggatggccgcattgct

SEQ ID NO: 25 - DNA, 48 bp, Homo sapiens
tggaatttgaaatatccgggggcctctacagaatcctggcatcagtta

SEQ ID NO: 26 - DNA, 15 bp, Homo sapiens
attttagctcctact

SEQ ID NO: 27 - DNA, 17 bp, Homo sapiens
tttagctcctactcaga

SEQ ID NO: 28 - DNA, 16 bp, Homo sapiens
agctcctactcagact

SEQ ID NO: 29 - DNA, 15 bp, Homo sapiens
cctactcagactgtt

SEQ ID NO: 30 - DNA, 17 bp, Homo sapiens
aaccacaggttgtgtca

SEQ ID NO: 31 - DNA, 16 bp, Homo sapiens
agtaaccacaggttgt

SEQ ID NO: 32 - DNA, 17 bp, Homo sapiens
ccttagtaaccacaggt

SEQ ID NO: 33 - DNA, 17 bp, Homo sapiens
gcaaaaacccaaaatat

SEQ ID NO: 34 - DNA, 17 bp, Homo sapiens
ttgcaaaaacccaaaat

SEQ ID NO: 35 - DNA, 17 bp, Homo sapiens
cctttttgcaaaaaccc

SEQ ID NO: 36 - DNA, 17 bp, Homo sapiens
caccagagtaacagtct

SEQ ID NO: 37 - DNA, 19 bp, Homo sapiens
gtcaccagagtaacagtct

SEQ ID NO: 38 - DNA, 18 bp, Homo sapiens
ccaaactagaaatgccat

SEQ ID NO: 39 - DNA, 19 bp, Homo sapiens
gaaatctgccagagcaggt

SEQ ID NO: 40 - DNA, 18 bp, Homo sapiens
ctatagatgagattatct

SEQ ID NO: 41 - DNA, 18 bp, Homo sapiens
agcaatgcggccatccct

SEQ ID NO: 42 - DNA, 17 bp, Homo sapiens
taactgatgccaggatt

SEQ ID NO: 43 - DNA, 17 bp, Homo sapiens
tggaatttgaaatatcc

SEQ ID NO: 44 - DNA, 48 bp, Artificial Sequence
  Synthetic
  misc_feature (18)..(31): n is a, c, g, or t
tggaatttgaaatatccnnnnnnnnnnnnnnaatcctggcatcagtta

SEQ ID NO: 45 - DNA, 48 bp, Mus musculus
tggaatttgaaatatccagaggcctctacagaatcctggcatcagtta

SEQ ID NO: 46 - DNA, 55 bp, Homo sapiens
tattttagctcctactcagactgttactctggtgacacaacctgtggttactaag

SEQ ID NO: 47 - protein, 8 aa, Homo sapiens
LLLRLLLW

SEQ ID NO: 48 - protein, 14 aa, Homo sapiens
SYSDCYSGDTTCGY

SEQ ID NO: 49 - protein, 15 aa, Homo sapiens
PTQTVTLVTQPVVTK

SEQ ID NO: 50 - DNA, 56 bp, Artificial Sequence
  Synthetic
  misc_feature (27)..(27): n is a, c, g, or t
tattttagctcctactcagactgttanctctggtgacacaacctgtggttactaag

SEQ ID NO: 51 - protein, 16 aa, Artificial Sequence
  Synthetic
  misc_feature (7)..(7): Xaa can be any naturally occurring amino acid
LLLRLLXLVTQPVVTK

SEQ ID NO: 52 - DNA, 57 bp, Artificial Sequence
  Synthetic
  misc_feature (27)..(28): n is a, c, g, or t
tattttagctcctactcagactgttannctctggtgacacaacctgtggttactaag

SEQ ID NO: 53 - protein, 16 aa, Artificial Sequence
  Synthetic
  misc_feature (6)..(7): Xaa can be any naturally occurring amino acid
SYSDCXXLVTQPVVTK

SEQ ID NO: 54 - DNA, 15 bp, Homo sapiens
attttagctcctact

SEQ ID NO: 55 - DNA, 17 bp, Homo sapiens
tttagctcctactcaga

SEQ ID NO: 56 - DNA, 16 bp, Homo sapiens
agctcctactcagact

SEQ ID NO: 57 - DNA, 15 bp, Homo sapiens
cctactcagactgtt

SEQ ID NO: 58 - DNA, 61 bp, Homo sapiens
aaaatattttagctcctactcagactgttactctggtgacacaacctgtggttactaagga

SEQ ID NO: 59 - DNA, 61 bp, Homo sapiens
tccttagtaaccacaggttgtgtcaccagagtaacagtctgagtaggagctaaaatatttt

SEQ ID NO: 60 - DNA, 25 bp, Artificial Sequence
  Synthetic
gagtttggctcaaattgttactctt

SEQ ID NO: 61 - DNA, 25 bp, Artificial Sequence
  Synthetic
gggaaatggtctaggagagtaaagt

SEQ ID NO: 62 - DNA, 34 bp, Artificial Sequence
  Synthetic
agactgttactcttggtgacacaacctgtgttac

SEQ ID NO: 63 - DNA, 59 bp, Homo sapiens
aaaaacccaaaatattttagctcctactcagactgttactctggtgacacaacctgtgg

SEQ ID NO: 64 - DNA, 56 bp, Artificial Sequence
  Synthetic
aaaaacccaaaatattttagctcctactcagactgttactgtgacacaacctgtgg

SEQ ID NO: 65 - DNA, 38 bp, Artificial Sequence
  Synthetic
aaaaacccaaaatattttagctcctactcagactgtgg

SEQ ID NO: 66 - DNA, 57 bp, Artificial Sequence
  Synthetic
aaaaacccaaaatattttagctcctactcagactgttactcttgacacaacctgtgg

SEQ ID NO: 67 - DNA, 49 bp, Artificial Sequence
  Synthetic
aaaacccaaaatattttagctcctactcagactgttacacaacctgtgg

SEQ ID NO: 68 - DNA, 57 bp, Artificial Sequence
  Synthetic
aaaaacccaaaatattttagctcctactcagactgttactggtgacacaacctgtgg

SEQ ID NO: 69 - DNA, 241 bp, Artificial Sequence
  Synthetic
  misc_feature (42)..(224): n is a, c, g, or t
aaaaacccaaaatattttagctcctactcagactgttactcnnnnnnnnnnnnnnnnnnnnnnnnnnnnnnnnnnnnnnnnnnnnnnnnnnnnnnnnnnnnnnnnnnnnnnnnnnnnnnnnnnnnnnnnnnnnnnnnnnnnnnnnnnnnnnnnnnnnnnnnnnnnnnnnnnnnnnnnnnnnnnnnnnnnnnnnnnnnnnnnnnnnnnnnnnnnnnnnnnnnnnnggtgacacaacctgtgg

SEQ ID NO: 70 - DNA, 57 bp, Artificial Sequence
  Synthetic
aaaaccccaaaattttttagctccttctcagactttttctggtgacacaacctgtgg

SEQ ID NO: 71 - DNA, 60 bp, Artificial Sequence
  Synthetic
aaaaacccaaaatattttagctcctactcagactgttactcttggtgacacaacctgtgg

SEQ ID NO: 72 - DNA, 53 bp, Artificial Sequence
  Synthetic
aaaaacccaaaatattttagctcctactcagactgttactctgcaacctgtgg

SEQ ID NO: 73 - DNA, 56 bp, Artificial Sequence
  Synthetic
aaaaacccaaaatattttagctcctactcagactgttacggtgacacaacctgtgg

SEQ ID NO: 74 - DNA, 59 bp, Artificial Sequence; identical to SEQ ID NO: 63
  Synthetic

SEQ ID NO: 75 - DNA, 34 bp, Homo sapiens
agactgttactctggtgacacaacctgtggttac

SEQ ID NO: 76 - DNA, 30 bp, Artificial Sequence
  Synthetic
agactgtttggtgacacaacctgtggttac

SEQ ID NO: 77 - DNA, 33 bp, Artificial Sequence
  Synthetic
agactgttactctgtgacacaacctgtggttac

SEQ ID NO: 78 - DNA, 25 bp, Artificial Sequence
  Synthetic
agactgtgacacaacctgtggttac

SEQ ID NO: 79 - DNA, 29 bp, Artificial Sequence
  Synthetic
agactgttactgacacaacctgtggttac

SEQ ID NO: 80 - DNA, 31 bp, Artificial Sequence
  Synthetic
agactgttactctgacacaacctgtggttac

SEQ ID NO: 81 - DNA, 31 bp, Artificial Sequence
  Synthetic
agactgttactgtgacacaacctgtggttac

SEQ ID NO: 82 - DNA, 31 bp, Artificial Sequence; identical to SEQ ID NO: 80
  Synthetic

SEQ ID NO: 83 - DNA, 34 bp, Homo sapiens; identical to SEQ ID NO: 75

SEQ ID NO: 84 - DNA, 31 bp, Artificial Sequence; identical to SEQ ID NO: 81
  Synthetic

SEQ ID NO: 85 - DNA, 13 bp, Artificial Sequence
  Synthetic
agactgtggttac

SEQ ID NO: 86 - DNA, 32 bp, Artificial Sequence
  Synthetic
agactgttactcttgacacaacctgtggttac

SEQ ID NO: 87 - DNA, 25 bp, Artificial Sequence
  Synthetic
agactgttacacaacctgtggttac

SEQ ID NO: 88 - DNA, 32 bp, Artificial Sequence
  Synthetic
agactgttactggtgacacaacctgtggttac

SEQ ID NO: 89 - DNA, 216 bp, Artificial Sequence
  Synthetic
  misc_feature (13)..(195): n is a, c, g, or t
agactgttactcnnnnnnnnnnnnnnnnnnnnnnnnnnnnnnnnnnnnnnnnnnnnnnnnnnnnnnnnnnnnnnnnnnnnnnnnnnnnnnnnnnnnnnnnnnnnnnnnnnnnnnnnnnnnnnnnnnnnnnnnnnnnnnnnnnnnnnnnnnnnnnnnnnnnnnnnnnnnnnnnnnnnnnnnnnnnnnnnnnnnnnnggtgacacaacctgtggttac

SEQ ID NO: 90 - DNA, 32 bp, Artificial Sequence; identical to SEQ ID NO: 88
  Synthetic

SEQ ID NO: 91 - DNA, 28 bp, Artificial Sequence
  Synthetic
agactgttactctgcaacctgtggttac

SEQ ID NO: 92 - DNA, 31 bp, Artificial Sequence
  Synthetic
agactgttacggtgacacaacctgtggttac

SEQ ID NO: 93 - DNA, 33 bp, Homo sapiens
agactgttactctggtgacacaacctgtgttac